European Patent Application EP 4 332 237 A1, published March 6, 2024. Title: ISOTHERMAL GENE AMPLIFICATION METHODS, GENE DETECTION METHODS, VIRUS DETECTION METHODS, AND KITS USED THEREWITH. Applicant: BioSeeds Corporation. The sequence listing filed with the application follows.

SEQUENCE LISTING (22 sequences)

SEQ ID NO: 1 - DNA, 28 bp, Bacteriophage T7
aattctaatacgactcactatagggaga

SEQ ID NO: 2 - DNA, 20 bp, Bacteriophage SP6
atttaggtgacactatagaa

SEQ ID NO: 3 - DNA, 120 bp, Artificial Sequence
  primer
aaaatgaaagatctcagtccaagatggtatttctactacctaggaactgggccagaagctggacttccctatggtgctaacaaagacggcatcatatgggttgcaactgagggagccttg

SEQ ID NO: 4 - DNA, 200 bp, Artificial Sequence
  primer
ttgcaactgagggagccttgaatacaccaaaagatcacattggcacccgcaatcctgctaacaatgctgcaatcgtgctacaacttcctcaaggaacaacattgccaaaaggcttctacgcagaagggagcagaggcggcagtcaagcctcttctcgttcctcatcacgtagtcgcaacagttcaagaaattcaactcca

SEQ ID NO: 5 - DNA, 120 bp, Artificial Sequence
  primer
tgctctcaagctggttcaatctgtcaagcagcagcaaagcaagagcagcatcaccgccattgccagccattctagcaggagaagttcccctactgctgcctggagttgaatttcttgaac

SEQ ID NO: 6 - DNA, 134 bp, Artificial Sequence
  target sequence
cacattggcacccgcaatcctgctaacaatgctgcaatcgtgctacaacttcctcaaggaacaacattgccaaaaggcttctacgcagaagggagcagaggcggcagtcaagcctcttctcgttcctctctccc

SEQ ID NO: 7 - DNA, 19 bp, Artificial Sequence
  primer
cacattggcacccgcaatc

SEQ ID NO: 8 - DNA, 48 bp, Artificial Sequence
  primer
aattctaatacgactcactatagggagagaggaacgagaagaggcttg

SEQ ID NO: 9 - DNA, 47 bp, Artificial Sequence
  primer
aattctaatacgactcactatagggagacacattggcacccgcaatc

SEQ ID NO: 10 - DNA, 20 bp, Artificial Sequence
  primer
gaggaacgagaagaggcttg

SEQ ID NO: 11 - DNA, 19 bp, Artificial Sequence
  primer
cacattggcacccgcaatc

SEQ ID NO: 12 - DNA, 20 bp, Artificial Sequence
  primer
gaggaacgagaagaggcttg

SEQ ID NO: 13 - DNA, 135 bp, Artificial Sequence
  target sequence
ttttccgacgtgctcgaactttttgggcatggaatcctgaggttaatgcaatcactgtcacaaccgtgttgggacagacatactatcaacccattcaacaagctccaacaggcattactgtgaccttgttgagcg

SEQ ID NO: 14 - DNA, 160 bp, Artificial Sequence
  primer
gctaattgggactctaattgggcctttgttgcatttagcttccttatggccgtatcaacactcgttatgtgggtgatgtactttgcaaatagtttcagacttttccgacgtgctcgaactttttgggcatggaatcctgaggttaatgcaatcactgtca

SEQ ID NO: 15 - DNA, 160 bp, Artificial Sequence
  primer
gtattcaggtaggttatgaacctgaacacctgaagccaatctatgtccgtcaacgtaaagcacgccgctcaacaaggtcacagtaatgcctgttggagcttgttgaatgggttgatagtatgtctgtcccaacacggttgtgacagtgattgcattaacc

SEQ ID NO: 16 - DNA, 25 bp, Artificial Sequence
  primer
ttttccgacgtgctcgaactttttg

SEQ ID NO: 17 - DNA, 53 bp, Artificial Sequence
  primer
aattctaatacgactcactatagggagacgctcaacaaggtcacagtaatgcc

SEQ ID NO: 18 - DNA, 203 bp, Artificial Sequence
  target sequence
ggccttcgggttgtaaagtactttcagcggggaggaagggagtaaagttaatacctttgctcattgacgttacccgcagaagaagcaccggctaactccgtgccagagccgcggtaatacggagggtgcaagcgttaatcggaattactgggcgtaaagcgcacgcaggcggtttgttaagtcagatgtgaaatccccgggct

SEQ ID NO: 19 - DNA, 19 bp, Artificial Sequence
  primer
agcccggggatttcacatc

SEQ ID NO: 20 - DNA, 49 bp, Artificial Sequence
  primer
aattctaatacgactcactatagggagaggccttcgggttgtaaagtac

SEQ ID NO: 21 - DNA, 28 bp, Artificial Sequence
  primer
ggccttcgggttgtaaagtactttcagc

SEQ ID NO: 22 - DNA, 26 bp, Artificial Sequence
  primer
agcccggggatttcacatctgactta